European Patent Application EP 4 180 522 A1, published May 17, 2023. Title: EXPRESSION CASSETTE FOR EXPRESSING GENE COMPRISING OVERLAPPING OPEN READING FRAMES IN INSECT CELL AND APPLICATION THEREOF. Applicant: GENEVOYAGER (WUHAN) CO., LTD. The sequence listing filed with the application follows.

SEQUENCE LISTING (46 sequences)

SEQ ID NO: 1 - DNA, 110 bp, AcMNPV
gacctttaattcaacccaacacaatatattatagttaaataagaattattatcaaatcatttgtatattaattaaaatactatactgtaaattacattttatttacaatc

SEQ ID NO: 2 - DNA, 137 bp, Artificial Sequence
  Intron
gtaagtattcattgtaaatctgatattatttgtattattatacctacctaatttgcagtgcagataaatatgccggatttatcgtgttcgccattagggcagtatattctcattcttccttttcctttttttttcag

SEQ ID NO: 3 - DNA, 108 bp, Artificial Sequence
  Intron
gtaagtatcgataactttgttttctttcacatttacaactccgacatacaaattcaggtatggcccattacggcagtataaattcgttcattttggatattgtttcag

SEQ ID NO: 4 - DNA, 110 bp, Artificial Sequence
  Intron
gtatcgataactttgttttctttcacatctacaacgccgacgccgccatggccatcgtgttcgccattagggcagtatattctcattcttccttttcctttttttttcag

SEQ ID NO: 5 - DNA, 179 bp, Artificial Sequence
  Intron
gtaagtattcattgtaaatctgatattatttgtattattatacctacctaatttgcagtgcagataaatatgccggatggtaattttattactgtttggtccataaacacttgtttaccatttccttttttacaagttttaatatgttctgcatatataaaacattatgtattttgcag

SEQ ID NO: 6 - DNA, 54 bp, Thosea asigna virus
gaagggcggggaagcctcctaacctgcggtgacgttgaggaaaatccgggtcca

SEQ ID NO: 7 - DNA, 2211 bp, Artificial Sequence
  Cap ORF
atggctgccgacggttatctacccgattggctcgaggacaaccttagtgaaggaattcgcgagtggtgggctttgaaacctggagcccctcaacccaaggcaaatcaacaacatcaagacaacgctcgaggtcttgtgcttccgggttacaaataccttggacccggcaacggactcgacaagggggagccggtcaacgcagcagacgcggcggccctcgagcacgacaaggcctacgaccagcagctcaaggccggagacaacccgtacctcaagtacaaccacgccgacgccgagttccaggagcggctcaaagaagatacgtcttttgggggcaacctcgggcgagcagtcttccaggccaaaaagaggcttcttgaacctcttggtctggttgaggaagcggctaagacggctcctggaaagaagaggcctgtagagcagtctcctcaggaaccggactcctccgcgggtattggcaaatcgggtgcacagcccgctaaaaagagactcaatttcggtcagactggcgacacagagtcagtcccagaccctcaaccaatcggagaacctcccgcagccccctcaggtgtgggatctcttacaatggcttcaggtggtggcgcaccagtggcagacaataacgaaggtgccgatggagtgggtagttcctcgggaaattggcattgcgattcccaatggctgggggacagagtcatcaccaccagcacccgaacctgggccctgcccacctacaacaatcacctctacaagcaaatctccaacagcacatctggaggatcttcaaatgacaacgcctacttcggctacagcaccccctgggggtattttgacttcaacagattccactgccacttctcaccacgtgactggcagcgactcatcaacaacaactggggattccggcctaagcgactcaacttcaagctcttcaacattcaggtcaaagaggttacggacaacaatggagtcaagaccatcgccaataaccttaccagcacggtccaggtcttcacggactcagactatcagctcccgtacgtgctcgggtcggctcacgagggctgcctcccgccgttcccagcggacgttttcatgattcctcagtacgggtatctgacgcttaatgatggaagccaggccgtgggtcgttcgtccttttactgcctggaatatttcccgtcgcaaatgctaagaacgggtaacaacttccagttcagctacgagtttgagaacgtacctttccatagcagctacgctcacagccaaagcctggaccgactaatgaatccactcatcgaccaatacttgtactatctctcaaagactattaacggttctggacagaatcaacaaacgctaaaattcagtgtggccggacccagcaacatggctgtccagggaagaaactacatacctggacccagctaccgacaacaacgtgtctcaaccactgtgactcaaaacaacaacagcgaatttgcttggcctggagcttcttcttgggctctcaatggacgtaatagcttgatgaatcctggacctgctatggccagccacaaagaaggagaggaccgtttctttcctttgtctggatctttaatttttggcaaacaaggaactggaagagacaacgtggatgcggacaaagtcatgataaccaacgaagaagaaattaaaactactaacccggtagcaacggagtcctatggacaagtggccacaaaccaccagagtgcccaagcacaggcgcagaccggctgggttcaaaaccaaggaatacttccgggtatggtttggcaggacagagatgtgtacctgcaaggacccatttgggccaaaattcctcacacggacggcaactttcacccttctccgctgatgggagggtttggaatgaagcacccgcctcctcagatcctcatcaaaaacacacctgtacctgcggatcctccaacggccttcaacaaggacaagctgaactctttcatcacccagtattctactggccaagtcagcgtggagatcgagtgggagctgcagaaggaaaacagcaagcgctggaacccggagatccagtacacttccaactattacaagtctaataatgttgaatttgctgttaatactgaaggtgtatatagtgaaccccgccccattggcaccagatacctgactcgtaatctgtaa

SEQ ID NO: 8 - DNA, 2566 bp, Artificial Sequence
  Cap gene expression cassette
gacctttaattcaacccaacacaatatattatagttaaataagaattattatcaaatcatttgtatattaattaaaatactatactgtaaattacattttatttacaatcactcgacgaagacttgatcacccgggtaggacaaggtaagtattcattgtaaatctgatattatttgtattattatacctacctaatttgcagtgcagataaatatgccggatttatcgtgttcgccattagggcagtatattctcattcttccttttcctttttttttcaggttcaccttcaacggctcgggagaagggcggggaagcctcctaacctgcggtgacgttgaggaaaatccgggtccagctgccgacggttatctacccgattggctcgaggacaaccttagtgaaggaattcgcgagtggtgggctttgaaacctggagcccctcaacccaaggcaaatcaacaacatcaagacaacgctcgaggtcttgtgcttccgggttacaaataccttggacccggcaacggactcgacaagggggagccggtcaacgcagcagacgcggcggccctcgagcacgacaaggcctacgaccagcagctcaaggccggagacaacccgtacctcaagtacaaccacgccgacgccgagttccaggagcggctcaaagaagatacgtcttttgggggcaacctcgggcgagcagtcttccaggccaaaaagaggcttcttgaacctcttggtctggttgaggaagcggctaagacggctcctggaaagaagaggcctgtagagcagtctcctcaggaaccggactcctccgcgggtattggcaaatcgggtgcacagcccgctaaaaagagactcaatttcggtcagactggcgacacagagtcagtcccagaccctcaaccaatcggagaacctcccgcagccccctcaggtgtgggatctcttacaatggcttcaggtggtggcgcaccagtggcagacaataacgaaggtgccgatggagtgggtagttcctcgggaaattggcattgcgattcccaatggctgggggacagagtcatcaccaccagcacccgaacctgggccctgcccacctacaacaatcacctctacaagcaaatctccaacagcacatctggaggatcttcaaatgacaacgcctacttcggctacagcaccccctgggggtattttgacttcaacagattccactgccacttctcaccacgtgactggcagcgactcatcaacaacaactggggattccggcctaagcgactcaacttcaagctcttcaacattcaggtcaaagaggttacggacaacaatggagtcaagaccatcgccaataaccttaccagcacggtccaggtcttcacggactcagactatcagctcccgtacgtgctcgggtcggctcacgagggctgcctcccgccgttcccagcggacgttttcatgattcctcagtacgggtatctgacgcttaatgatggaagccaggccgtgggtcgttcgtccttttactgcctggaatatttcccgtcgcaaatgctaagaacgggtaacaacttccagttcagctacgagtttgagaacgtacctttccatagcagctacgctcacagccaaagcctggaccgactaatgaatccactcatcgaccaatacttgtactatctctcaaagactattaacggttctggacagaatcaacaaacgctaaaattcagtgtggccggacccagcaacatggctgtccagggaagaaactacatacctggacccagctaccgacaacaacgtgtctcaaccactgtgactcaaaacaacaacagcgaatttgcttggcctggagcttcttcttgggctctcaatggacgtaatagcttgatgaatcctggacctgctatggccagccacaaagaaggagaggaccgtttctttcctttgtctggatctttaatttttggcaaacaaggaactggaagagacaacgtggatgcggacaaagtcatgataaccaacgaagaagaaattaaaactactaacccggtagcaacggagtcctatggacaagtggccacaaaccaccagagtgcccaagcacaggcgcagaccggctgggttcaaaaccaaggaatacttccgggtatggtttggcaggacagagatgtgtacctgcaaggacccatttgggccaaaattcctcacacggacggcaactttcacccttctccgctgatgggagggtttggaatgaagcacccgcctcctcagatcctcatcaaaaacacacctgtacctgcggatcctccaacggccttcaacaaggacaagctgaactctttcatcacccagtattctactggccaagtcagcgtggagatcgagtgggagctgcagaaggaaaacagcaagcgctggaacccggagatccagtacacttccaactattacaagtctaataatgttgaatttgctgttaatactgaaggtgtatatagtgaaccccgccccattggcaccagatacctgactcgtaatctgtaa

SEQ ID NO: 9 - DNA, 2529 bp, Artificial Sequence
  Cap gene expression cassette
gacctttaattcaacccaacacaatatattatagttaaataagaattattatcaaatcatttgtatattaattaaaatactatactgtaaattacattttatttacaatcactcgacgaagacttgatcacccgggcagcaggtaagtatcgataactttgttttctttcacatttacaactccgacatacaaattcaggtatggcccattacggcagtataaattcgttcattttggatattgtttcagttgcaagtggctcgggagaagggcggggaagcctcctaacctgcggtgacgttgaggaaaatccgggtccagctgccgacggttatcttcccgattggctcgaggacaaccttagtgaaggaattcgcgagtggtgggctttgaaacctggagcccctcaacccaaggcaaatcaacaacatcaagacaacgctcgaggtcttgtgcttccgggttacaaataccttggacccggcaacggactcgacaagggggagccggtcaacgcagcagacgcggcggccctcgagcacgacaaggcctacgaccagcagctcaaggccggagacaacccgtacctcaagtacaaccacgccgacgccgagttccaggagcggctcaaagaagatacgtcttttgggggcaacctcgggcgagcagtcttccaggccaaaaagaggcttcttgaacctcttggtctggttgaggaagcggctaagacggctcctggaaagaagaggcctgtagagcagtctcctcaggaaccggactcctccgcgggtattggcaaatcgggtgcacagcccgctaaaaagagactcaatttcggtcagactggcgacacagagtcagtcccagaccctcaaccaatcggagaacctcccgcagccccctcaggtgtgggatctcttacaatggcttcaggtggtggcgcaccagtggcagacaataacgaaggtgccgatggagtgggtagttcctcgggaaattggcattgcgattcccaatggctgggggacagagtcatcaccaccagcacccgaacctgggccctgcccacctacaacaatcacctctacaagcaaatctccaacagcacatctggaggatcttcaaatgacaacgcctacttcggctacagcaccccctgggggtattttgacttcaacagattccactgccacttctcaccacgtgactggcagcgactcatcaacaacaactggggattccggcctaagcgactcaacttcaagctcttcaacattcaggtcaaagaggttacggacaacaatggagtcaagaccatcgccaataaccttaccagcacggtccaggtcttcacggactcagactatcagctcccgtacgtgctcgggtcggctcacgagggctgcctcccgccgttcccagcggacgttttcatgattcctcagtacgggtatctgacgcttaatgatggaagccaggccgtgggtcgttcgtccttttactgcctggaatatttcccgtcgcaaatgctaagaacgggtaacaacttccagttcagctacgagtttgagaacgtacctttccatagcagctacgctcacagccaaagcctggaccgactaatgaatccactcatcgaccaatacttgtactatctctcaaagactattaacggttctggacagaatcaacaaacgctaaaattcagtgtggccggacccagcaacatggctgtccagggaagaaactacatacctggacccagctaccgacaacaacgtgtctcaaccactgtgactcaaaacaacaacagcgaatttgcttggcctggagcttcttcttgggctctcaatggacgtaatagcttgatgaatcctggacctgctatggccagccacaaagaaggagaggaccgtttctttcctttgtctggatctttaatttttggcaaacaaggaactggaagagacaacgtggatgcggacaaagtcatgataaccaacgaagaagaaattaaaactactaacccggtagcaacggagtcctatggacaagtggccacaaaccaccagagtgcccaagcacaggcgcagaccggctgggttcaaaaccaaggaatacttccgggtatggtttggcaggacagagatgtgtacctgcaaggacccatttgggccaaaattcctcacacggacggcaactttcacccttctccgctgatgggagggtttggaatgaagcacccgcctcctcagatcctcatcaaaaacacacctgtacctgcggatcctccaacggccttcaacaaggacaagctgaactctttcatcacccagtattctactggccaagtcagcgtggagatcgagtgggagctgcagaaggaaaacagcaagcgctggaacccggagatccagtacacttccaactattacaagtctaataatgttgaatttgctgttaatactgaaggtgtatatagtgaaccccgccccattggcaccagatacctgactcgtaatctgtaa

SEQ ID NO: 10 - DNA, 2527 bp, Artificial Sequence
  Cap gene expression cassette
gacctttaattcaacccaacacaatatattatagttaaataagaattattatcaaatcatttgtatattaattaaaatactatactgtaaattacattttatttacaatcactcgacgaagacttgatcacccgggcaggtaagtatcgataactttgttttctttcacatctacaacgccgacgccgccatggccatcgtgttcgccattagggcagtatattctcattcttccttttcctttttttttcaggttggctcgggagaagggcggggaagcctcctaacctgcggtgacgttgaggaaaatccgggtccagctgccgacggttatctacccgattggctcgaggacaaccttagtgaaggaattcgcgagtggtgggctttgaaacctggagcccctcaacccaaggcaaatcaacaacatcaagacaacgctcgaggtcttgtgcttccgggttacaaataccttggacccggcaacggactcgacaagggggagccggtcaacgcagcagacgcggcggccctcgagcacgacaaggcctacgaccagcagctcaaggccggagacaacccgtacctcaagtacaaccacgccgacgccgagttccaggagcggctcaaagaagatacgtcttttgggggcaacctcgggcgagcagtcttccaggccaaaaagaggcttcttgaacctcttggtctggttgaggaagcggctaagacggctcctggaaagaagaggcctgtagagcagtctcctcaggaaccggactcctccgcgggtattggcaaatcgggtgcacagcccgctaaaaagagactcaatttcggtcagactggcgacacagagtcagtcccagaccctcaaccaatcggagaacctcccgcagccccctcaggtgtgggatctcttacaatggcttcaggtggtggcgcaccagtggcagacaataacgaaggtgccgatggagtgggtagttcctcgggaaattggcattgcgattcccaatggctgggggacagagtcatcaccaccagcacccgaacctgggccctgcccacctacaacaatcacctctacaagcaaatctccaacagcacatctggaggatcttcaaatgacaacgcctacttcggctacagcaccccctgggggtattttgacttcaacagattccactgccacttctcaccacgtgactggcagcgactcatcaacaacaactggggattccggcctaagcgactcaacttcaagctcttcaacattcaggtcaaagaggttacggacaacaatggagtcaagaccatcgccaataaccttaccagcacggtccaggtcttcacggactcagactatcagctcccgtacgtgctcgggtcggctcacgagggctgcctcccgccgttcccagcggacgttttcatgattcctcagtacgggtatctgacgcttaatgatggaagccaggccgtgggtcgttcgtccttttactgcctggaatatttcccgtcgcaaatgctaagaacgggtaacaacttccagttcagctacgagtttgagaacgtacctttccatagcagctacgctcacagccaaagcctggaccgactaatgaatccactcatcgaccaatacttgtactatctctcaaagactattaacggttctggacagaatcaacaaacgctaaaattcagtgtggccggacccagcaacatggctgtccagggaagaaactacatacctggacccagctaccgacaacaacgtgtctcaaccactgtgactcaaaacaacaacagcgaatttgcttggcctggagcttcttcttgggctctcaatggacgtaatagcttgatgaatcctggacctgctatggccagccacaaagaaggagaggaccgtttctttcctttgtctggatctttaatttttggcaaacaaggaactggaagagacaacgtggatgcggacaaagtcatgataaccaacgaagaagaaattaaaactactaacccggtagcaacggagtcctatggacaagtggccacaaaccaccagagtgcccaagcacaggcgcagaccggctgggttcaaaaccaaggaatacttccgggtatggtttggcaggacagagatgtgtacctgcaaggacccatttgggccaaaattcctcacacggacggcaactttcacccttctccgctgatgggagggtttggaatgaagcacccgcctcctcagatcctcatcaaaaacacacctgtacctgcggatcctccaacggccttcaacaaggacaagctgaactctttcatcacccagtattctactggccaagtcagcgtggagatcgagtgggagctgcagaaggaaaacagcaagcgctggaacccggagatccagtacacttccaactattacaagtctaataatgttgaatttgctgttaatactgaaggtgtatatagtgaaccccgccccattggcaccagatacctgactcgtaatctgtaa

SEQ ID NO: 11 - DNA, 2605 bp, Artificial Sequence
  Cap gene expression cassette
gacctttaattcaacccaacacaatatattatagttaaataagaattattatcaaatcatttgtatattaattaaaatactatactgtaaattacattttatttacaatcactcgacgaagacttgatcacccgggtaggacaaggtaagtattcattgtaaatctgatattatttgtattattatacctacctaatttgcagtgcagataaatatgccggatggtaattttattactgtttggtccataaacacttgtttaccatttccttttttacaagttttaatatgttctgcatatataaaacattatgtattttgcagcaccttcaacggctcgggagaagggcggggaagcctcctaacctgcggtgacgttgaggaaaatccgggtccagctgccgacggttatctacccgattggctcgaggacaaccttagtgaaggaattcgcgagtggtgggctttgaaacctggagcccctcaacccaaggcaaatcaacaacatcaagacaacgctcgaggtcttgtgcttccgggttacaaataccttggacccggcaacggactcgacaagggggagccggtcaacgcagcagacgcggcggccctcgagcacgacaaggcctacgaccagcagctcaaggccggagacaacccgtacctcaagtacaaccacgccgacgccgagttccaggagcggctcaaagaagatacgtcttttgggggcaacctcgggcgagcagtcttccaggccaaaaagaggcttcttgaacctcttggtctggttgaggaagcggctaagacggctcctggaaagaagaggcctgtagagcagtctcctcaggaaccggactcctccgcgggtattggcaaatcgggtgcacagcccgctaaaaagagactcaatttcggtcagactggcgacacagagtcagtcccagaccctcaaccaatcggagaacctcccgcagccccctcaggtgtgggatctcttacaatggcttcaggtggtggcgcaccagtggcagacaataacgaaggtgccgatggagtgggtagttcctcgggaaattggcattgcgattcccaatggctgggggacagagtcatcaccaccagcacccgaacctgggccctgcccacctacaacaatcacctctacaagcaaatctccaacagcacatctggaggatcttcaaatgacaacgcctacttcggctacagcaccccctgggggtattttgacttcaacagattccactgccacttctcaccacgtgactggcagcgactcatcaacaacaactggggattccggcctaagcgactcaacttcaagctcttcaacattcaggtcaaagaggttacggacaacaatggagtcaagaccatcgccaataaccttaccagcacggtccaggtcttcacggactcagactatcagctcccgtacgtgctcgggtcggctcacgagggctgcctcccgccgttcccagcggacgttttcatgattcctcagtacgggtatctgacgcttaatgatggaagccaggccgtgggtcgttcgtccttttactgcctggaatatttcccgtcgcaaatgctaagaacgggtaacaacttccagttcagctacgagtttgagaacgtacctttccatagcagctacgctcacagccaaagcctggaccgactaatgaatccactcatcgaccaatacttgtactatctctcaaagactattaacggttctggacagaatcaacaaacgctaaaattcagtgtggccggacccagcaacatggctgtccagggaagaaactacatacctggacccagctaccgacaacaacgtgtctcaaccactgtgactcaaaacaacaacagcgaatttgcttggcctggagcttcttcttgggctctcaatggacgtaatagcttgatgaatcctggacctgctatggccagccacaaagaaggagaggaccgtttctttcctttgtctggatctttaatttttggcaaacaaggaactggaagagacaacgtggatgcggacaaagtcatgataaccaacgaagaagaaattaaaactactaacccggtagcaacggagtcctatggacaagtggccacaaaccaccagagtgcccaagcacaggcgcagaccggctgggttcaaaaccaaggaatacttccgggtatggtttggcaggacagagatgtgtacctgcaaggacccatttgggccaaaattcctcacacggacggcaactttcacccttctccgctgatgggagggtttggaatgaagcacccgcctcctcagatcctcatcaaaaacacacctgtacctgcggatcctccaacggccttcaacaaggacaagctgaactctttcatcacccagtattctactggccaagtcagcgtggagatcgagtgggagctgcagaaggaaaacagcaagcgctggaacccggagatccagtacacttccaactattacaagtctaataatgttgaatttgctgttaatactgaaggtgtatatagtgaaccccgccccattggcaccagatacctgactcgtaatctgtaa

SEQ ID NO: 12 - DNA, 92 bp, AcMNPV
atcatggagataattaaaatgataaccatctcgcaaataaataagtattttactgttttcgtaacagttttgtaataaaaaaacctataaat

SEQ ID NO: 13 - DNA, 1863 bp, Artificial Sequence
  Rep ORF
atggggttttacgagattgtgattaaggtccccagcgaccttgacgggcatctgcccggcatttctgacagctttgtgaactgggtggccgagaaggagtgggagttgccgccagattctgacttggatctgaatctgattgagcaggcacccctgaccgtggccgagaagctgcagcgcgactttctgacggagtggcgccgtgtgagtaaggccccggaggcccttttctttgtgcaatttgagaagggagagagctacttccacttacacgtgctcgtggaaaccaccggggtgaaatccttagttttgggacgtttcctgagtcagattcgcgaaaaactgattcagagaatttaccgcgggatcgagccgactttgccaaactggttcgcggtcacaaagaccagaaacggcgccggaggcgggaacaaggtggtggacgagtgctacatccccaattacttgctccccaaaacccagcctgagctccagtgggcgtggactaatttagaacagtatttaagcgcctgtttgaatctcacggagcgtaaacggttggtggcgcagcatctgacgcacgtgtcgcagacgcaggagcagaacaaagagaatcagaatcccaattctgacgcgccggtgatcagatcaaaaacttcagccaggtacatggagctggtcgggtggctcgtggacaaggggattacctcggagaagcagtggatccaggaggaccaggcctcatacatctccttcaatgcggcctccaactcgcggtcccaaatcaaggctgccttggacaatgcgggaaagattatgagcctgactaaaaccgcccccgactacctggtgggccagcagcccgtggaggacatttccagcaatcggatttataaaattttggaactaaacgggtacgatccccaatatgcggcttccgtctttctgggatgggccacgaaaaagttcggcaagaggaacaccatctggctgtttgggcctgcaactaccgggaagaccaacatcgcggaggccatagcccacactgtgcccttctacgggtgcgtaaactggaccaatgagaactttcccttcaacgactgtgtcgacaagatggtgatctggtgggaggaggggaagatgaccgccaaggtcgtggagtcggccaaagccattctcggaggaagcaaggtgcgcgtggaccagaaatgcaagtcctcggcccagatagacccgactcccgtgatcgtcacctccaacaccaacatgtgcgccgtgattgacgggaactcaacgaccttcgaacaccagcagccgttgcaagaccggatgttcaaatttgaactcacccgccgtctggatcatgactttgggaaggtcaccaagcaggaagtcaaagactttttccggtgggcaaaggatcacgtggttgaggtggagcatgaattctacgtcaaaaagggtggagccaagaaaagacccgcccccagtgacgcagatataagtgagcccaaacgggtgcgcgagtcagttgcgcagccatcgacgtcagacgcggaagcttcgatcaactacgcagacaggtaccaaaacaaatgttctcgtcacgtgggcatgaatctgatgctgtttccctgcagacaatgcgagagaatgaatcagaattcaaatatctgcttcactcacggacagaaagactgtttagagtgctttcccgtgtcagaatctcaacccgtttctgtcgtcaaaaaggcgtatcagaaactgtgctacattcatcatatcatgggaaaggtgccagacgcttgcactgcctgcgatctggtcaatgtggatttggatgactgcatctttgaacaataa

SEQ ID NO: 14 - DNA, 2255 bp, Artificial Sequence
  Rep gene expression cassette
atcatggagataattaaaatgataaccatctcgcaaataaataagtattttactgttttcgtaacagttttgtaataaaaaaacctataaatattccggattattcataccgtcccaccatcgggcgcggatcctaggacaaggtaagtatgcattgtaaatgtgatattatgtgtattattatacctacctaatttgcagtgcagataaatatgccggatggtaattttattactgtttggtccataaacacttgtttaccatttccttttttacaagttttaatatgttctgcatatataaaacattatgtattttgcagcaccttcaacggctcgggagaagggcggggaagcctcctaacctgcggtgacgttgaggaaaatccgggtccagggttttacgagattgtgattaaggtccccagcgaccttgacgggcatctgcccggcatttctgacagctttgtgaactgggtggccgagaaggagtgggagttgccgccagattctgacttggatctgaatctgattgagcaggcacccctgaccgtggccgagaagctgcagcgcgactttctgacggagtggcgccgtgtgagtaaggccccggaggcccttttctttgtgcaatttgagaagggagagagctacttccacttacacgtgctcgtggaaaccaccggggtgaaatccttagttttgggacgtttcctgagtcagattcgcgaaaaactgattcagagaatttaccgcgggatcgagccgactttgccaaactggttcgcggtcacaaagaccagaaacggcgccggaggcgggaacaaggtggtggacgagtgctacatccccaattacttgctccccaaaacccagcctgagctccagtgggcgtggactaatttagaacagtatttaagcgcctgtttgaatctcacggagcgtaaacggttggtggcgcagcatctgacgcacgtgtcgcagacgcaggagcagaacaaagagaatcagaatcccaattctgacgcgccggtgatcagatcaaaaacttcagccaggtacatggagctggtcgggtggctcgtggacaaggggattacctcggagaagcagtggatccaggaggaccaggcctcatacatctccttcaatgcggcctccaactcgcggtcccaaatcaaggctgccttggacaatgcgggaaagattatgagcctgactaaaaccgcccccgactacctggtgggccagcagcccgtggaggacatttccagcaatcggatttataaaattttggaactaaacgggtacgatccccaatatgcggcttccgtctttctgggatgggccacgaaaaagttcggcaagaggaacaccatctggctgtttgggcctgcaactaccgggaagaccaacatcgcggaggccatagcccacactgtgcccttctacgggtgcgtaaactggaccaatgagaactttcccttcaacgactgtgtcgacaagatggtgatctggtgggaggaggggaagatgaccgccaaggtcgtggagtcggccaaagccattctcggaggaagcaaggtgcgcgtggaccagaaatgcaagtcctcggcccagatagacccgactcccgtgatcgtcacctccaacaccaacatgtgcgccgtgattgacgggaactcaacgaccttcgaacaccagcagccgttgcaagaccggatgttcaaatttgaactcacccgccgtctggatcatgactttgggaaggtcaccaagcaggaagtcaaagactttttccggtgggcaaaggatcacgtggttgaggtggagcatgaattctacgtcaaaaagggtggagccaagaaaagacccgcccccagtgacgcagatataagtgagcccaaacgggtgcgcgagtcagttgcgcagccatcgacgtcagacgcggaagcttcgatcaactacgcagacaggtaccaaaacaaatgttctcgtcacgtgggcatgaatctgatgctgtttccctgcagacaatgcgagagaatgaatcagaattcaaatatctgcttcactcacggacagaaagactgtttagagtgctttcccgtgtcagaatctcaacccgtttctgtcgtcaaaaaggcgtatcagaaactgtgctacattcatcatatcatgggaaaggtgccagacgcttgcactgcctgcgatctggtcaatgtggatttggatgactgcatctttgaacaataa

SEQ ID NO: 15 - DNA, 226 bp, Artificial Sequence
  Intron
gtaagtatcgataactttgttttctttcacatttacaactccgacatacaaatgccgccatggtaagtattcattgtaaatctgatattatttgtattattatacctacctaatttgcagtgcagggtaattttattactgtttggtccataaacacttgtttaccatttccttttttacaagttttaatattttctgcatatataaaacattatttattttgcag

SEQ ID NO: 16 - DNA, 226 bp, Artificial Sequence
  Intron
gtaagtattcattgtaaatctgatattatttgtattattatacctacctaatttgcagtgcaggccgccatggtaagtatcgataactttgttttctttcacatttacaactccgacatacaaattgtaattttattactgtttggtccataaacacttgtttaccatttccttttttacaagttttaatattttctgcatatataaaacattatttattttgcag

SEQ ID NO: 17 - DNA, 2605 bp, Artificial Sequence; identical to SEQ ID NO: 11
  Cap gene expression cassette

SEQ ID NO: 18 - DNA, 2499 bp, Artificial Sequence
  Cap gene expression cassette
gacctttaattcaacccaacacaatatattatagttaaataagaattattatcaaatcatttgtatattaattaaaatactatactgtaaattacattttatttacaatcactcgacgaagacttgatcacccgggtagctaaaggtatttctttgactctaaaaaccttgacgactgtttcgccttgaacaaactaaatgaaccctttatgcaaacagctgcccgtgggctcgggagaagggcggggaagcctcctaacctgcggtgacgttgaggaaaatccgggtccagctgccgacggttatctacccgattggctcgaggacaaccttagtgaaggaattcgcgagtggtgggctttgaaacctggagcccctcaacccaaggcaaatcaacaacatcaagacaacgctcgaggtcttgtgcttccgggttacaaataccttggacccggcaacggactcgacaagggggagccggtcaacgcagcagacgcggcggccctcgagcacgacaaggcctacgaccagcagctcaaggccggagacaacccgtacctcaagtacaaccacgccgacgccgagttccaggagcggctcaaagaagatacgtcttttgggggcaacctcgggcgagcagtcttccaggccaaaaagaggcttcttgaacctcttggtctggttgaggaagcggctaagacggctcctggaaagaagaggcctgtagagcagtctcctcaggaaccggactcctccgcgggtattggcaaatcgggtgcacagcccgctaaaaagagactcaatttcggtcagactggcgacacagagtcagtcccagaccctcaaccaatcggagaacctcccgcagccccctcaggtgtgggatctcttacaatggcttcaggtggtggcgcaccagtggcagacaataacgaaggtgccgatggagtgggtagttcctcgggaaattggcattgcgattcccaatggctgggggacagagtcatcaccaccagcacccgaacctgggccctgcccacctacaacaatcacctctacaagcaaatctccaacagcacatctggaggatcttcaaatgacaacgcctacttcggctacagcaccccctgggggtattttgacttcaacagattccactgccacttctcaccacgtgactggcagcgactcatcaacaacaactggggattccggcctaagcgactcaacttcaagctcttcaacattcaggtcaaagaggttacggacaacaatggagtcaagaccatcgccaataaccttaccagcacggtccaggtcttcacggactcagactatcagctcccgtacgtgctcgggtcggctcacgagggctgcctcccgccgttcccagcggacgttttcatgattcctcagtacgggtatctgacgcttaatgatggaagccaggccgtgggtcgttcgtccttttactgcctggaatatttcccgtcgcaaatgctaagaacgggtaacaacttccagttcagctacgagtttgagaacgtacctttccatagcagctacgctcacagccaaagcctggaccgactaatgaatccactcatcgaccaatacttgtactatctctcaaagactattaacggttctggacagaatcaacaaacgctaaaattcagtgtggccggacccagcaacatggctgtccagggaagaaactacatacctggacccagctaccgacaacaacgtgtctcaaccactgtgactcaaaacaacaacagcgaatttgcttggcctggagcttcttcttgggctctcaatggacgtaatagcttgatgaatcctggacctgctatggccagccacaaagaaggagaggaccgtttctttcctttgtctggatctttaatttttggcaaacaaggaactggaagagacaacgtggatgcggacaaagtcatgataaccaacgaagaagaaattaaaactactaacccggtagcaacggagtcctatggacaagtggccacaaaccaccagagtgcccaagcacaggcgcagaccggctgggttcaaaaccaaggaatacttccgggtatggtttggcaggacagagatgtgtacctgcaaggacccatttgggccaaaattcctcacacggacggcaactttcacccttctccgctgatgggagggtttggaatgaagcacccgcctcctcagatcctcatcaaaaacacacctgtacctgcggatcctccaacggccttcaacaaggacaagctgaactctttcatcacccagtattctactggccaagtcagcgtggagatcgagtgggagctgcagaaggaaaacagcaagcgctggaacccggagatccagtacacttccaactattacaagtctaataatgttgaatttgctgttaatactgaaggtgtatatagtgaaccccgccccattggcaccagatacctgactcgtaatctgtaa

SEQ ID NO: 19 - DNA, 2224 bp, Artificial Sequence
  Rep gene expression cassette
atcatggagataattaaaatgataaccatctcgcaaataaataagtattttactgttttcgtaacagttttgtaataaaaaaacctataaatattccggattattcataccgtcccaccatcgggcgcggatccggacaaggtaagtattcattgtaaatctgatattatttgtattattatacctacctaatttgcagtgcaggccgccatggtaagtatcgataactttgttttctttcacatttacaactccgacatacaaattgtaattttattactgtttggtccataaacacttgtttaccatttccttttttacaagttttaatattttctgcatatataaaacattatttattttgcaggggttttacgagattgtgattaaggtccccagcgaccttgacgggcatctgcccggcatttctgacagctttgtgaactgggtggccgagaaggagtgggagttgccgccagattctgacttggatctgaatctgattgagcaggcacccctgaccgtggccgagaagctgcagcgcgactttctgacggagtggcgccgtgtgagtaaggccccggaggcccttttctttgtgcaatttgagaagggagagagctacttccacttacacgtgctcgtggaaaccaccggggtgaaatccttagttttgggacgtttcctgagtcagattcgcgaaaaactgattcagagaatttaccgcgggatcgagccgactttgccaaactggttcgcggtcacaaagaccagaaacggcgccggaggcgggaacaaggtggtggacgagtgctacatccccaattacttgctccccaaaacccagcctgagctccagtgggcgtggactaatttagaacagtatttaagcgcctgtttgaatctcacggagcgtaaacggttggtggcgcagcatctgacgcacgtgtcgcagacgcaggagcagaacaaagagaatcagaatcccaattctgacgcgccggtgatcagatcaaaaacttcagccaggtacatggagctggtcgggtggctcgtggacaaggggattacctcggagaagcagtggatccaggaggaccaggcctcatacatctccttcaatgcggcctccaactcgcggtcccaaatcaaggctgccttggacaatgcgggaaagattatgagcctgactaaaaccgcccccgactacctggtgggccagcagcccgtggaggacatttccagcaatcggatttataaaattttggaactaaacgggtacgatccccaatatgcggcttccgtctttctgggatgggccacgaaaaagttcggcaagaggaacaccatctggctgtttgggcctgcaactaccgggaagaccaacatcgcggaggccatagcccacactgtgcccttctacgggtgcgtaaactggaccaatgagaactttcccttcaacgactgtgtcgacaagatggtgatctggtgggaggaggggaagatgaccgccaaggtcgtggagtcggccaaagccattctcggaggaagcaaggtgcgcgtggaccagaaatgcaagtcctcggcccagatagacccgactcccgtgatcgtcacctccaacaccaacatgtgcgccgtgattgacgggaactcaacgaccttcgaacaccagcagccgttgcaagaccggatgttcaaatttgaactcacccgccgtctggatcatgactttgggaaggtcaccaagcaggaagtcaaagactttttccggtgggcaaaggatcacgtggttgaggtggagcatgaattctacgtcaaaaagggtggagccaagaaaagacccgcccccagtgacgcagatataagtgagcccaaacgggtgcgcgagtcagttgcgcagccatcgacgtcagacgcggaagcttcgatcaactacgcagacaggtaccaaaacaaatgttctcgtcacgtgggcatgaatctgatgctgtttccctgcagacaatgcgagagaatgaatcagaattcaaatatctgcttcactcacggacagaaagactgtttagagtgctttcccgtgtcagaatctcaacccgtttctgtcgtcaaaaaggcgtatcagaaactgtgctacattcatcatatcatgggaaaggtgccagacgcttgcactgcctgcgatctggtcaatgtggatttggatgactgcatctttgaacaa

SEQ ID NO: 20 - DNA, 98 bp, Artificial Sequence
  Intron
gtaagtatcgataactttgttttctttcacatttacaactccgacatacaaatcccattacggcagtataaattcgttcattttggatattgtttcag

SEQ ID NO: 21 - DNA, 108 bp, Artificial Sequence
  Intron
gtaagtattcattgtaaatctgatattatttgtattattatacctacctaatttgcagtgcagcccattacggcagtataaattcgttcattttggatattgtttcag

SEQ ID NO: 22 - DNA, 2451 bp, Artificial Sequence
  Cap gene expression cassette
gacctttaattcaacccaacacaatatattatagttaaataagaattattatcaaatcatttgtatattaattaaaatactatactgtaaattacattttatttacaatcactcgacgaagacttgatcacccgggtcaggtagtaagtatcgataactttgttttctttcacatttacaactccgacatacaaatcccattacggcagtataaattcgttcattttggatattgtttcagtggctgccgacggttatctacccgattggctcgaggacaaccttagtgaaggaattcgcgagtggtgggctttgaaacctggagcccctcaacccaaggcaaatcaacaacatcaagacaacgctcgaggtcttgtgcttccgggttacaaataccttggacccggcaacggactcgacaagggggagccggtcaacgcagcagacgcggcggccctcgagcacgacaaggcctacgaccagcagctcaaggccggagacaacccgtacctcaagtacaaccacgccgacgccgagttccaggagcggctcaaagaagatacgtcttttgggggcaacctcgggcgagcagtcttccaggccaaaaagaggcttcttgaacctcttggtctggttgaggaagcggctaagacggctcctggaaagaagaggcctgtagagcagtctcctcaggaaccggactcctccgcgggtattggcaaatcgggtgcacagcccgctaaaaagagactcaatttcggtcagactggcgacacagagtcagtcccagaccctcaaccaatcggagaacctcccgcagccccctcaggtgtgggatctcttacaatggcttcaggtggtggcgcaccagtggcagacaataacgaaggtgccgatggagtgggtagttcctcgggaaattggcattgcgattcccaatggctgggggacagagtcatcaccaccagcacccgaacctgggccctgcccacctacaacaatcacctctacaagcaaatctccaacagcacatctggaggatcttcaaatgacaacgcctacttcggctacagcaccccctgggggtattttgacttcaacagattccactgccacttctcaccacgtgactggcagcgactcatcaacaacaactggggattccggcctaagcgactcaacttcaagctcttcaacattcaggtcaaagaggttacggacaacaatggagtcaagaccatcgccaataaccttaccagcacggtccaggtcttcacggactcagactatcagctcccgtacgtgctcgggtcggctcacgagggctgcctcccgccgttcccagcggacgttttcatgattcctcagtacgggtatctgacgcttaatgatggaagccaggccgtgggtcgttcgtccttttactgcctggaatatttcccgtcgcaaatgctaagaacgggtaacaacttccagttcagctacgagtttgagaacgtacctttccatagcagctacgctcacagccaaagcctggaccgactaatgaatccactcatcgaccaatacttgtactatctctcaaagactattaacggttctggacagaatcaacaaacgctaaaattcagtgtggccggacccagcaacatggctgtccagggaagaaactacatacctggacccagctaccgacaacaacgtgtctcaaccactgtgactcaaaacaacaacagcgaatttgcttggcctggagcttcttcttgggctctcaatggacgtaatagcttgatgaatcctggacctgctatggccagccacaaagaaggagaggaccgtttctttcctttgtctggatctttaatttttggcaaacaaggaactggaagagacaacgtggatgcggacaaagtcatgataaccaacgaagaagaaattaaaactactaacccggtagcaacggagtcctatggacaagtggccacaaaccaccagagtgcccaagcacaggcgcagaccggctgggttcaaaaccaaggaatacttccgggtatggtttggcaggacagagatgtgtacctgcaaggacccatttgggccaaaattcctcacacggacggcaactttcacccttctccgctgatgggagggtttggaatgaagcacccgcctcctcagatcctcatcaaaaacacacctgtacctgcggatcctccaacggccttcaacaaggacaagctgaactctttcatcacccagtattctactggccaagtcagcgtggagatcgagtgggagctgcagaaggaaaacagcaagcgctggaacccggagatccagtacacttccaactattacaagtctaataatgttgaatttgctgttaatactgaaggtgtatatagtgaaccccgccccattggcaccagatacctgactcgtaatctgtaa

SEQ ID NO: 23 - DNA, 2461 bp, Artificial Sequence
  Cap gene expression cassette
gacctttaattcaacccaacacaatatattatagttaaataagaattattatcaaatcatttgtatattaattaaaatactatactgtaaattacattttatttacaatcactcgacgaagacttgatcacccggggccgccagtaagtattcattgtaaatctgatattatttgtattattatacctacctaatttgcagtgcagcccattacggcagtataaattcgttcattttggatattgtttcagtggctgccgacggttatctacccgattggctcgaggacaaccttagtgaaggaattcgcgagtggtgggctttgaaacctggagcccctcaacccaaggcaaatcaacaacatcaagacaacgctcgaggtcttgtgcttccgggttacaaataccttggacccggcaacggactcgacaagggggagccggtcaacgcagcagacgcggcggccctcgagcacgacaaggcctacgaccagcagctcaaggccggagacaacccgtacctcaagtacaaccacgccgacgccgagttccaggagcggctcaaagaagatacgtcttttgggggcaacctcgggcgagcagtcttccaggccaaaaagaggcttcttgaacctcttggtctggttgaggaagcggctaagacggctcctggaaagaagaggcctgtagagcagtctcctcaggaaccggactcctccgcgggtattggcaaatcgggtgcacagcccgctaaaaagagactcaatttcggtcagactggcgacacagagtcagtcccagaccctcaaccaatcggagaacctcccgcagccccctcaggtgtgggatctcttacaatggcttcaggtggtggcgcaccagtggcagacaataacgaaggtgccgatggagtgggtagttcctcgggaaattggcattgcgattcccaatggctgggggacagagtcatcaccaccagcacccgaacctgggccctgcccacctacaacaatcacctctacaagcaaatctccaacagcacatctggaggatcttcaaatgacaacgcctacttcggctacagcaccccctgggggtattttgacttcaacagattccactgccacttctcaccacgtgactggcagcgactcatcaacaacaactggggattccggcctaagcgactcaacttcaagctcttcaacattcaggtcaaagaggttacggacaacaatggagtcaagaccatcgccaataaccttaccagcacggtccaggtcttcacggactcagactatcagctcccgtacgtgctcgggtcggctcacgagggctgcctcccgccgttcccagcggacgttttcatgattcctcagtacgggtatctgacgcttaatgatggaagccaggccgtgggtcgttcgtccttttactgcctggaatatttcccgtcgcaaatgctaagaacgggtaacaacttccagttcagctacgagtttgagaacgtacctttccatagcagctacgctcacagccaaagcctggaccgactaatgaatccactcatcgaccaatacttgtactatctctcaaagactattaacggttctggacagaatcaacaaacgctaaaattcagtgtggccggacccagcaacatggctgtccagggaagaaactacatacctggacccagctaccgacaacaacgtgtctcaaccactgtgactcaaaacaacaacagcgaatttgcttggcctggagcttcttcttgggctctcaatggacgtaatagcttgatgaatcctggacctgctatggccagccacaaagaaggagaggaccgtttctttcctttgtctggatctttaatttttggcaaacaaggaactggaagagacaacgtggatgcggacaaagtcatgataaccaacgaagaagaaattaaaactactaacccggtagcaacggagtcctatggacaagtggccacaaaccaccagagtgcccaagcacaggcgcagaccggctgggttcaaaaccaaggaatacttccgggtatggtttggcaggacagagatgtgtacctgcaaggacccatttgggccaaaattcctcacacggacggcaactttcacccttctccgctgatgggagggtttggaatgaagcacccgcctcctcagatcctcatcaaaaacacacctgtacctgcggatcctccaacggccttcaacaaggacaagctgaactctttcatcacccagtattctactggccaagtcagcgtggagatcgagtgggagctgcagaaggaaaacagcaagcgctggaacccggagatccagtacacttccaactattacaagtctaataatgttgaatttgctgttaatactgaaggtgtatatagtgaaccccgccccattggcaccagatacctgactcgtaatctgtaa

SEQ ID NO: 24 - DNA, 2111 bp, Artificial Sequence
  Rep gene expression cassette
atcatggagataattaaaatgataaccatctcgcaaataaataagtattttactgttttcgtaacagttttgtaataaaaaaacctataaatattccggattattcataccgtcccaccatcgggcgcggatcctcaggtagtaagtattcattgtaaatctgatattatttgtattattatacctacctaatttgcagtgcagcccattacggcagtataaattcgttcattttggatattgtttcagtggggttttacgagattgtgattaaggtccccagcgaccttgacgggcatctgcccggcatttctgacagctttgtgaactgggtggccgagaaggagtgggagttgccgccagattctgacttggatctgaatctgattgagcaggcacccctgaccgtggccgagaagctgcagcgcgactttctgacggagtggcgccgtgtgagtaaggccccggaggcccttttctttgtgcaatttgagaagggagagagctacttccacttacacgtgctcgtggaaaccaccggggtgaaatccttagttttgggacgtttcctgagtcagattcgcgaaaaactgattcagagaatttaccgcgggatcgagccgactttgccaaactggttcgcggtcacaaagaccagaaacggcgccggaggcgggaacaaggtggtggacgagtgctacatccccaattacttgctccccaaaacccagcctgagctccagtgggcgtggactaatttagaacagtatttaagcgcctgtttgaatctcacggagcgtaaacggttggtggcgcagcatctgacgcacgtgtcgcagacgcaggagcagaacaaagagaatcagaatcccaattctgacgcgccggtgatcagatcaaaaacttcagccaggtacatggagctggtcgggtggctcgtggacaaggggattacctcggagaagcagtggatccaggaggaccaggcctcatacatctccttcaatgcggcctccaactcgcggtcccaaatcaaggctgccttggacaatgcgggaaagattatgagcctgactaaaaccgcccccgactacctggtgggccagcagcccgtggaggacatttccagcaatcggatttataaaattttggaactaaacgggtacgatccccaatatgcggcttccgtctttctgggatgggccacgaaaaagttcggcaagaggaacaccatctggctgtttgggcctgcaactaccgggaagaccaacatcgcggaggccatagcccacactgtgcccttctacgggtgcgtaaactggaccaatgagaactttcccttcaacgactgtgtcgacaagatggtgatctggtgggaggaggggaagatgaccgccaaggtcgtggagtcggccaaagccattctcggaggaagcaaggtgcgcgtggaccagaaatgcaagtcctcggcccagatagacccgactcccgtgatcgtcacctccaacaccaacatgtgcgccgtgattgacgggaactcaacgaccttcgaacaccagcagccgttgcaagaccggatgttcaaatttgaactcacccgccgtctggatcatgactttgggaaggtcaccaagcaggaagtcaaagactttttccggtgggcaaaggatcacgtggttgaggtggagcatgaattctacgtcaaaaagggtggagccaagaaaagacccgcccccagtgacgcagatataagtgagcccaaacgggtgcgcgagtcagttgcgcagccatcgacgtcagacgcggaagcttcgatcaactacgcagacaggtaccaaaacaaatgttctcgtcacgtgggcatgaatctgatgctgtttccctgcagacaatgcgagagaatgaatcagaattcaaatatctgcttcactcacggacagaaagactgtttagagtgctttcccgtgtcagaatctcaacccgtttctgtcgtcaaaaaggcgtatcagaaactgtgctacattcatcatatcatgggaaaggtgccagacgcttgcactgcctgcgatctggtcaatgtggatttggatgactgcatctttgaacaataa

SEQ ID NO: 25 - DNA, 2048 bp, Artificial Sequence
  Cap gene expression cassette
atacggacctttaattcaacccaacacaatatattatagttaaataagaattattatcaaatcatttgtatattaattaaaatactatactgtaaattacattttatttacaatcactcgacgaagacttgatcacccggggctaagacggctgccgacggttatctacccgattggctcgaggacaaccttagtgaaggaattcgcgagtggtgggctttgaaacctggagcccctcaacccaaggcaaatcaacaacatcaagacaacgctcgaggtcttgtgcttccgggttacaaataccttggacccggcaacggactcgacaagggggagccggtcaacgcagcagacgcggcggccctcgagcacgacaaggcctacgaccagcagctcaaggccggagacaacccgtacctcaagtacaaccacgccgacgccgagttccaggagcggctcaaagaagatacgtcttttgggggcaacctcgggcgagcagtcttccaggccaaaaagaggcttcttgaacctcttggtctggttgaggaagcggctaagacggctcctggaaagaagaggcctgtagagcagtctcctcaggaaccggactcctccgcgggtattggcaaatcgggtgcacagcccgctaaaaagagactcaatttcggtcagactggcgacacagagtcagtcccagaccctcaaccaatcggagaacctcccgcagccccctcaggtgtgggatctcttacaatggcttcaggtggtggcgcaccagtggcagacaataacgaaggtgccgatggagtgggtagttcctcgggaaattggcattgcgattcccaatggctgggggacagagtcatcaccaccagcacccgaacctgggccctgcccacctacaacaatcacctctacaagcaaatctccaacagcacatctggaggatcttcaaatgacaacgcctacttcggctacagcaccccctgggggtattttgacttcaacagattccactgccacttctcaccacgtgactggcagcgactcatcaacaacaactggggattccggcctaagcgactcaacttcaagctcttcaacattcaggtcaaagaggttacggacaacaatggagtcaagaccatcgccaataaccttaccagcacggtccaggtcttcacggactcagactatcagctcccgtacgtgctcgggtcggctcacgagggctgcctcccgccgttcccagcggacgttttcatgattcctcagtacgggtatctgacgcttaatgatggaagccaggccgtgggtcgttcgtccttttactgcctggaatatttcccgtcgcaaatgctaagaacgggtaacaacttccagttcagctacgagtttgagaacgtacctttccatagcagctacgctcacagccaaagcctggaccgactaatgaatccactcatcgaccaatacttgtactatctctcaaagactattaacggttctggacagaatcaacaaacgctaaaattcagtgtggccggacccagcaacatggctgtccagggaagaaactacatacctggacccagctaccgacaacaacgtgtctcaaccactgtgactcaaaacaacaacagcgaatttgcttggcctggagcttcttcttgggctctcaatggacgtaatagcttgatgaatcctggacctgctatggccagccacaaagaaggagaggaccgtttctttcctttgtctggatctttaatttttggcaaacaaggaactggaagagacaacgtggatgcggacaaagtcatgataaccaacgaagaagaaattaaaactactaacccggtagcaacggagtcctatggacaagtggccacaaaccaccagagtgcccaagcacaggcgcagaccggctgggttcaaaaccaaggaatacttccgggtatggtttggcaggacagagatgtgtacctgcaaggacccatttgggccaaaattcctcacacggacggcaactttcacccttctccgct

SEQ ID NO: 26 - DNA, 4814 bp, Artificial Sequence
  ITR -GOI
cctgcaggcagctgcgcgctcgctcgctcactgaggccgcccgggcaaagcccgggcgtcgggcgacctttggtcgcccggcctcagtgagcgagcgagcgcgcagagagggagtggccaactccatcactaggggttcctgcggccgcacgcgccgcccgtcagtgggcagagcgcacatcgcccacagtccccgagaagttggggggaggggtcggcaattgaaccggtgcctagagaaggtggcgcggggtaaactgggaaagtgatgtcgtgtactggctccgcctttttcccgagggtgggggagaaccgtatataagtgcagtagtcgccgtgaacgttctttttcgcaacgggtttgccgccagaacacgcgtaagggatccgccaccatggtgagcaagggcgaggaggataacatggccatcatcaaggagttcatgcgcttcaaggtgcacatggagggctccgtgaacggccacgagttcgagatcgagggcgagggcgagggccgcccctacgagggcacccagaccgccaagctgaaggtgaccaagggtggccccctgcccttcgcctgggacatcctgtcccctcagttcatgtacggctccaaggcctacgtgaagcaccccgccgacatccccgactacttgaagctgtccttccccgagggcttcaagtgggagcgcgtgatgaacttcgaggacggcggcgtggtgaccgtgacccaggactcctccctgcaggacggcgagttcatctacaaggtgaagctgcgcggcaccaacttcccctccgacggccccgtaatgcagaagaagaccatgggctgggaggcctcctccgagcggatgtaccccgaggacggcgccctgaagggcgagatcaagcagaggctgaagctgaaggacggcggccactacgacgctgaggtcaagaccacctacaaggccaagaagcccgtgcagctgcccggcgcctacaacgtcaacatcaagttggacatcacctcccacaacgaggactacaccatcgtggaacagtacgaacgcgccgagggccgccactccaccggcggcatggacgagctgtacaagtaagaattcgatatcaagcttatcgataatcaacctctggattacaaaatttgtgaaagattgactggtattcttaactatgttgctccttttacgctatgtggatacgctgctttaatgcctttgtatcatgctattgcttcccgtatggctttcattttctcctccttgtataaatcctggttgctgtctctttatgaggagttgtggcccgttgtcaggcaacgtggcgtggtgtgcactgtgtttgctgacgcaacccccactggttggggcattgccaccacctgtcagctcctttccgggactttcgctttccccctccctattgccacggcggaactcatcgccgcctgccttgcccgctgctggacaggggctcggctgttgggcactgacaattccgtggtgttgtcggggaaatcatcgtcctttccttggctgctcgcctgtgttgccacctggattctgcgcgggacgtccttctgctacgtcccttcggccctcaatccagcggaccttccttcccgcggcctgctgccggctctgcggcctcttccgcgtcttcgccttcgccctcagacgagtcggatctccctttgggccgcctccccgcatcgataccgagcgctgctcgagagatctacgggtggcatccctgtgacccctccccagtgcctctcctggccctggaagttgccactccagtgcccaccagccttgtcctaataaaattaagttgcatcattttgtctgactaggtgtccttctataatattatggggtggaggggggtggtatggagcaaggggcaagttgggaagacaacctgtagggcctgcggggtctattgggaaccaagctggagtgcagtggcacaatcttggctcactgcaatctccgcctcctgggttcaagcgattctcctgcctcagcctcccgagttgttgggattccaggcatgcatgaccaggctcagctaatttttgtttttttggtagagacggggtttcaccatattggccaggctggtctccaactcctaatctcaggtgatctacccaccttggcctcccaaattgctgggattacaggcgtgaaccactgctcccttccctgtccttctgattttgtaggtaaccacgtgcggaccgagcggccgcaggaacccctagtgatggagttggccactccctctctgcgcgctcgctcgctcactgaggccgggcgaccaaaggtcgcccgacgcccgggctttgcccgggcggcctcagtgagcgagcgagcgcgcagctgcctgcaggcctgcaggcagctgcgcgctcgctcgctcactgaggccgcccgggcaaagcccgggcgtcgggcgacctttggtcgcccggcctcagtgagcgagcgagcgcgcagagagggagtggccaactccatcactaggggttcctgcggccgcacgcgccgcccgtcagtgggcagagcgcacatcgcccacagtccccgagaagttggggggaggggtcggcaattgaaccggtgcctagagaaggtggcgcggggtaaactgggaaagtgatgtcgtgtactggctccgcctttttcccgagggtgggggagaaccgtatataagtgcagtagtcgccgtgaacgttctttttcgcaacgggtttgccgccagaacacgcgtaagggatccgccaccatggtgagcaagggcgaggaggataacatggccatcatcaaggagttcatgcgcttcaaggtgcacatggagggctccgtgaacggccacgagttcgagatcgagggcgagggcgagggccgcccctacgagggcacccagaccgccaagctgaaggtgaccaagggtggccccctgcccttcgcctgggacatcctgtcccctcagttcatgtacggctccaaggcctacgtgaagcaccccgccgacatccccgactacttgaagctgtccttccccgagggcttcaagtgggagcgcgtgatgaacttcgaggacggcggcgtggtgaccgtgacccaggactcctccctgcaggacggcgagttcatctacaaggtgaagctgcgcggcaccaacttcccctccgacggccccgtaatgcagaagaagaccatgggctgggaggcctcctccgagcggatgtaccccgaggacggcgccctgaagggcgagatcaagcagaggctgaagctgaaggacggcggccactacgacgctgaggtcaagaccacctacaaggccaagaagcccgtgcagctgcccggcgcctacaacgtcaacatcaagttggacatcacctcccacaacgaggactacaccatcgtggaacagtacgaacgcgccgagggccgccactccaccggcggcatggacgagctgtacaagtaagaattcgatatcaagcttatcgataatcaacctctggattacaaaatttgtgaaagattgactggtattcttaactatgttgctccttttacgctatgtggatacgctgctttaatgcctttgtatcatgctattgcttcccgtatggctttcattttctcctccttgtataaatcctggttgctgtctctttatgaggagttgtggcccgttgtcaggcaacgtggcgtggtgtgcactgtgtttgctgacgcaacccccactggttggggcattgccaccacctgtcagctcctttccgggactttcgctttccccctccctattgccacggcggaactcatcgccgcctgccttgcccgctgctggacaggggctcggctgttgggcactgacaattccgtggtgttgtcggggaaatcatcgtcctttccttggctgctcgcctgtgttgccacctggattctgcgcgggacgtccttctgctacgtcccttcggccctcaatccagcggaccttccttcccgcggcctgctgccggctctgcggcctcttccgcgtcttcgccttcgccctcagacgagtcggatctccctttgggccgcctccccgcatcgataccgagcgctgctcgagagatctacgggtggcatccctgtgacccctccccagtgcctctcctggccctggaagttgccactccagtgcccaccagccttgtcctaataaaattaagttgcatcattttgtctgactaggtgtccttctataatattatggggtggaggggggtggtatggagcaaggggcaagttgggaagacaacctgtagggcctgcggggtctattgggaaccaagctggagtgcagtggcacaatcttggctcactgcaatctccgcctcctgggttcaagcgattctcctgcctcagcctcccgagttgttgggattccaggcatgcatgaccaggctcagctaatttttgtttttttggtagagacggggtttcaccatattggccaggctggtctccaactcctaatctcaggtgatctacccaccttggcctcccaaattgctgggattacaggcgtgaaccactgctcccttccctgtccttctgattttgtaggtaaccacgtgcggaccgagcggccgcaggaacccctagtgatggagttggccactccctctctgcgcgctcgctcgctcactgaggccgggcgaccaaaggtcgcccgacgcccgggctttgcccgggcggcctcagtgagcgagcgagcgcgcagctgcctgcagg

SEQ ID NO: 27 - DNA, 2602 bp, Artificial Sequence
  Cap gene expression cassette
gacctttaattcaacccaacacaatatattatagttaaataagaattattatcaaatcatttgtatattaattaaaatactatactgtaaattacattttatttacaatcactcgacgaagacttgatcacccgggtaggacaaggtaagtattcattgtaaatctgatattatttgtattattatacctacctaatttgcagtgcagataaatatgccggatggtaattttattactgtttggtccataaacacttgtttaccatttccttttttacaagttttaatatgttctgcatatataaaacattatgtattttgcagcaccttcaacggctcgggagaagggcggggaagcctcctaacctgcggtgacgttgaggaaaatccgggtccagctgccgacggttatctacccgattggctcgaggacactctctctgaaggaataagacagtggtggaagctcaaacctggcccaccaccaccaaagcccgcagagcggcataaggacgacagcaggggtcttgtgcttcctgggtacaagtacctcggacccttcaacggactcgacaagggagagccggtcaacgaggcagacgccgcggccctcgagcacgacaaagcctacgaccggcagctcgacagcggagacaacccgtacctcaagtacaaccacgccgacgcggagtttcaggagcgccttaaagaagatacgtcttttgggggcaacctcggacgagcagtcttccaggcgaaaaagagggttcttgaacctctgggcctggttgaggaacctgttaagacggctccgggaaaaaagaggccggtagagcactctcctgtggagccagactcctcctcgggaaccggaaaggcgggccagcagcctgcaagaaaaagattgaattttggtcagactggagacgcagactcagtacctgacccccagcctctcggacagccaccagcagccccctctggtctgggaactaatacgatggctacaggcagtggcgcaccaatggcagacaataacgagggcgccgacggagtgggtaattcctcgggaaattggcattgcgattccacatggatgggcgacagagtcatcaccaccagcacccgaacctgggccctgcccacctacaacaaccacctctacaaacaaatttccagccaatcaggagcctcgaacgacaatcactactttggctacagcaccccttgggggtattttgacttcaacagattccactgccacttttcaccacgtgactggcaaagactcatcaacaacaactggggattccgacccaagagactcaacttcaagctctttaacattcaagtcaaagaggtcacgcagaatgacggtacgacgacgattgccaataaccttaccagcacggttcaggtgtttactgactcggagtaccagctcccgtacgtcctcggctcggcgcatcaaggatgcctcccgccgttcccagcagacgtcttcatggtgccacagtatggatacctcaccctgaacaacgggagtcaggcagtaggacgctcttcattttactgcctggagtactttccttctcagatgctgcgtaccggaaacaactttaccttcagctacacttttgaggacgttcctttccacagcagctacgctcacagccagagtctggaccgtctcatgaatcctctcatcgaccagtacctgtattacttgagcagaacaaacactccaagtggaaccaccacgcagtcaaggcttcagttttctcaggccggagcgagtgacattcgggaccagtctaggaactggcttcctggaccctgttaccgccagcagcgagtatcaaagacatctgcggataacaacaacagtgaatactcgtggactggagctaccaagtaccacctcaatggcagagactctctggtgaatccgggcccggccatggcaagccacaaggacgatgaagaaaagttttttcctcagagcggggttctcatctttgggaagcaaggctcagagaaaacaaatgtggacattgaaaaggtcatgattacagacgaagaggaaatcaggacaaccaatcccgtggctacggagcagtatggttctgtatctaccaacctccagagaggcaacagacaagcagctaccgcagatgtcaacacacaaggcgttcttccaggcatggtctggcaggacagagatgtgtaccttcaggggcccatctgggcaaagattccacacacggacggacattttcacccctctcccctcatgggtggattcggacttaaacaccctcctccacagattctcatcaagaacaccccggtacctgcgaatccttcgaccaccttcagtgcggcaaagtttgcttccttcatcacacagtactccacgggacaggtcagcgtggagatcgagtgggagctgcagaaggaaaacagcaaacgctggaatcccgaaattcagtacacttccaactacaacaagtctgttaatgtggactttactgtggacactaatggcgtgtattcagagcctcgccccattggcaccagatacctgactcgtaatctgtaa

SEQ ID NO: 28 - DNA, 2574 bp, Artificial Sequence
  Cap gene expression cassette
gacctttaattcaacccaacacaatatattatagttaaataagaattattatcaaatcatttgtatattaattaaaatactatactgtaaattacattttatttacaatcactcgacgaagacttgatcacccgggggacaaggtaagtattcattgtaaatctgatattatttgtattattatacctacctaatttgcagtgcaggccgccatggtaagtatcgataactttgttttctttcacatttacaactccgacatacaaattgtaattttattactgtttggtccataaacacttgtttaccatttccttttttacaagttttaatattttctgcatatataaaacattatttattttgcaggctgccgacggttatctacccgattggctcgaggacactctctctgaaggaataagacagtggtggaagctcaaacctggcccaccaccaccaaagcccgcagagcggcataaggacgacagcaggggtcttgtgcttcctgggtacaagtacctcggacccttcaacggactcgacaagggagagccggtcaacgaggcagacgccgcggccctcgagcacgacaaagcctacgaccggcagctcgacagcggagacaacccgtacctcaagtacaaccacgccgacgcggagtttcaggagcgccttaaagaagatacgtcttttgggggcaacctcggacgagcagtcttccaggcgaaaaagagggttcttgaacctctgggcctggttgaggaacctgttaagacggctccgggaaaaaagaggccggtagagcactctcctgtggagccagactcctcctcgggaaccggaaaggcgggccagcagcctgcaagaaaaagattgaattttggtcagactggagacgcagactcagtacctgacccccagcctctcggacagccaccagcagccccctctggtctgggaactaatacgatggctacaggcagtggcgcaccaatggcagacaataacgagggcgccgacggagtgggtaattcctcgggaaattggcattgcgattccacatggatgggcgacagagtcatcaccaccagcacccgaacctgggccctgcccacctacaacaaccacctctacaaacaaatttccagccaatcaggagcctcgaacgacaatcactactttggctacagcaccccttgggggtattttgacttcaacagattccactgccacttttcaccacgtgactggcaaagactcatcaacaacaactggggattccgacccaagagactcaacttcaagctctttaacattcaagtcaaagaggtcacgcagaatgacggtacgacgacgattgccaataaccttaccagcacggttcaggtgtttactgactcggagtaccagctcccgtacgtcctcggctcggcgcatcaaggatgcctcccgccgttcccagcagacgtcttcatggtgccacagtatggatacctcaccctgaacaacgggagtcaggcagtaggacgctcttcattttactgcctggagtactttccttctcagatgctgcgtaccggaaacaactttaccttcagctacacttttgaggacgttcctttccacagcagctacgctcacagccagagtctggaccgtctcatgaatcctctcatcgaccagtacctgtattacttgagcagaacaaacactccaagtggaaccaccacgcagtcaaggcttcagttttctcaggccggagcgagtgacattcgggaccagtctaggaactggcttcctggaccctgttaccgccagcagcgagtatcaaagacatctgcggataacaacaacagtgaatactcgtggactggagctaccaagtaccacctcaatggcagagactctctggtgaatccgggcccggccatggcaagccacaaggacgatgaagaaaagttttttcctcagagcggggttctcatctttgggaagcaaggctcagagaaaacaaatgtggacattgaaaaggtcatgattacagacgaagaggaaatcaggacaaccaatcccgtggctacggagcagtatggttctgtatctaccaacctccagagaggcaacagacaagcagctaccgcagatgtcaacacacaaggcgttcttccaggcatggtctggcaggacagagatgtgtaccttcaggggcccatctgggcaaagattccacacacggacggacattttcacccctctcccctcatgggtggattcggacttaaacaccctcctccacagattctcatcaagaacaccccggtacctgcgaatccttcgaccaccttcagtgcggcaaagtttgcttccttcatcacacagtactccacgggacaggtcagcgtggagatcgagtgggagctgcagaaggaaaacagcaaacgctggaatcccgaaattcagtacacttccaactacaacaagtctgttaatgtggactttactgtggacactaatggcgtgtattcagagcctcgccccattggcaccagatacctgactcgtaatctgtaa

SEQ ID NO: 29 - DNA, 2448 bp, Artificial Sequence
  Cap gene expression cassette
gacctttaattcaacccaacacaatatattatagttaaataagaattattatcaaatcatttgtatattaattaaaatactatactgtaaattacattttatttacaatcactcgacgaagacttgatcacccgggtcaggtagtaagtatcgataactttgttttctttcacatttacaactccgacatacaaatcccattacggcagtataaattcgttcattttggatattgtttcagtggctgccgacggttatctacccgattggctcgaggacactctctctgaaggaataagacagtggtggaagctcaaacctggcccaccaccaccaaagcccgcagagcggcataaggacgacagcaggggtcttgtgcttcctgggtacaagtacctcggacccttcaacggactcgacaagggagagccggtcaacgaggcagacgccgcggccctcgagcacgacaaagcctacgaccggcagctcgacagcggagacaacccgtacctcaagtacaaccacgccgacgcggagtttcaggagcgccttaaagaagatacgtcttttgggggcaacctcggacgagcagtcttccaggcgaaaaagagggttcttgaacctctgggcctggttgaggaacctgttaagacggctccgggaaaaaagaggccggtagagcactctcctgtggagccagactcctcctcgggaaccggaaaggcgggccagcagcctgcaagaaaaagattgaattttggtcagactggagacgcagactcagtacctgacccccagcctctcggacagccaccagcagccccctctggtctgggaactaatacgatggctacaggcagtggcgcaccaatggcagacaataacgagggcgccgacggagtgggtaattcctcgggaaattggcattgcgattccacatggatgggcgacagagtcatcaccaccagcacccgaacctgggccctgcccacctacaacaaccacctctacaaacaaatttccagccaatcaggagcctcgaacgacaatcactactttggctacagcaccccttgggggtattttgacttcaacagattccactgccacttttcaccacgtgactggcaaagactcatcaacaacaactggggattccgacccaagagactcaacttcaagctctttaacattcaagtcaaagaggtcacgcagaatgacggtacgacgacgattgccaataaccttaccagcacggttcaggtgtttactgactcggagtaccagctcccgtacgtcctcggctcggcgcatcaaggatgcctcccgccgttcccagcagacgtcttcatggtgccacagtatggatacctcaccctgaacaacgggagtcaggcagtaggacgctcttcattttactgcctggagtactttccttctcagatgctgcgtaccggaaacaactttaccttcagctacacttttgaggacgttcctttccacagcagctacgctcacagccagagtctggaccgtctcatgaatcctctcatcgaccagtacctgtattacttgagcagaacaaacactccaagtggaaccaccacgcagtcaaggcttcagttttctcaggccggagcgagtgacattcgggaccagtctaggaactggcttcctggaccctgttaccgccagcagcgagtatcaaagacatctgcggataacaacaacagtgaatactcgtggactggagctaccaagtaccacctcaatggcagagactctctggtgaatccgggcccggccatggcaagccacaaggacgatgaagaaaagttttttcctcagagcggggttctcatctttgggaagcaaggctcagagaaaacaaatgtggacattgaaaaggtcatgattacagacgaagaggaaatcaggacaaccaatcccgtggctacggagcagtatggttctgtatctaccaacctccagagaggcaacagacaagcagctaccgcagatgtcaacacacaaggcgttcttccaggcatggtctggcaggacagagatgtgtaccttcaggggcccatctgggcaaagattccacacacggacggacattttcacccctctcccctcatgggtggattcggacttaaacaccctcctccacagattctcatcaagaacaccccggtacctgcgaatccttcgaccaccttcagtgcggcaaagtttgcttccttcatcacacagtactccacgggacaggtcagcgtggagatcgagtgggagctgcagaaggaaaacagcaaacgctggaatcccgaaattcagtacacttccaactacaacaagtctgttaatgtggactttactgtggacactaatggcgtgtattcagagcctcgccccattggcaccagatacctgactcgtaatctgtaa

SEQ ID NO: 30 - DNA, 2569 bp, Artificial Sequence
  Cap gene expression cassette
gacctttaattcaacccaacacaatatattatagttaaataagaattattatcaaatcatttgtatattaattaaaatactatactgtaaattacattttatttacaatcactcgacgaagacttgatcacccgggtaggacaaggtaagtattcattgtaaatctgatattatttgtattattatacctacctaatttgcagtgcagataaatatgccggatggtaattttattactgtttggtccataaacacttgtttaccatttccttttttacaagttttaatatgttctgcatatataaaacattatgtattttgcagcaccttcaacggctcgggagaagggcggggaagcctcctaacctgcggtgacgttgaggaaaatccgggtccatcttttgttgatcacccacccgattggttggaagaagttggtgaaggtcttcgcgagtttttgggccttgaagcgggcccaccgaaaccaaaacccaatcagcagcatcaagatcaagcccgtggtcttgtgctgcctggttataactatctcggacccggaaacggtctcgatcgaggagagcctgtcaacagggcagacgaggtcgcgcgagagcacgacatctcgtacaacgagcagcttgaggcgggagacaacccctacctcaagtacaaccacgcggacgccgagtttcaggagaagctcgccgacgacacatccttcgggggaaacctcggaaaggcagtctttcaggccaagaaaagggttctcgaaccttttggcctggttgaagagggtgctaagacggcccctaccggaaagcggatagacgaccactttccaaaaagaaagaaggctcggaccgaagaggactccaagccttccacctcgtcagacgccgaagctggacccagcggatcccagcagctgcaaatcccagcccaaccagcctcaagtttgggagctgatacaatgtctgcgggaggtggcggcccattgggcgacaataaccaaggtgccgatggagtgggcaatgcctcgggagattggcattgcgattccacgtggatgggggacagagtcgtcaccaagtccacccgaacctgggtgctgcccagctacaacaaccaccagtaccgagagatcaaaagcggctccgtcgacggaagcaacgccaacgcctactttggatacagcaccccctgggggtactttgactttaaccgcttccacagccactggagcccccgagactggcaaagactcatcaacaactactggggcttcagaccccggtccctcagagtcaaaatcttcaacattcaagtcaaagaggtcacggtgcaggactccaccaccaccatcgccaacaacctcacctccaccgtccaagtgtttacggacgacgactaccagctgccctacgtcgtcggcaacgggaccgagggatgcctgccggccttccctccgcaggtctttacgctgccgcagtacggttacgcgacgctgaaccgcgacaacacagaaaatcccaccgagaggagcagcttcttctgcctagagtactttcccagcaagatgctgagaacgggcaacaactttgagtttacctacaactttgaggaggtgcccttccactccagcttcgctcccagtcagaacctcttcaagctggccaacccgctggtggaccagtacttgtaccgcttcgtgagcacaaataacactggcggagtccagttcaacaagaacctggccgggagatacgccaacacctacaaaaactggttcccggggcccatgggccgaacccagggctggaacctgggctccggggtcaaccgcgccagtgtcagcgccttcgccacgaccaataggatggagctcgagggcgcgagttaccaggtgcccccgcagccgaacggcatgaccaacaacctccagggcagcaacacctatgccctggagaacactatgatcttcaacagccagccggcgaacccgggcaccaccgccacgtacctcgagggcaacatgctcatcaccagcgagagcgagacgcagccggtgaaccgcgtggcgtacaacgtcggcgggcagatggccaccaacaaccagagctccaccactgcccccgcgaccggcacgtacaacctccaggaaatcgtgcccggcagcgtgtggatggagagggacgtgtacctccaaggacccatctgggccaagatcccagagacgggggcgcactttcacccctctccggccatgggcggattcggactcaaacacccaccgcccatgatgctcatcaagaacacgcctgtgcccggaaatatcaccagcttctcggacgtgcccgtcagcagcttcatcacccagtacagcaccgggcaggtcaccgtggagatggagtgggagctcaagaaggaaaactccaagaggtggaacccagagatccagtacacaaacaactacaacgacccccagtttgtggactttgccccggacagcaccggggaatacagaagcaccagacctatcggaacccgataccttacccgacccctttaa

SEQ ID NO: 31 - DNA, 2541 bp, Artificial Sequence
  Cap gene expression cassette
gacctttaattcaacccaacacaatatattatagttaaataagaattattatcaaatcatttgtatattaattaaaatactatactgtaaattacattttatttacaatcactcgacgaagacttgatcacccgggggacaaggtaagtattcattgtaaatctgatattatttgtattattatacctacctaatttgcagtgcaggccgccatggtaagtatcgataactttgttttctttcacatttacaactccgacatacaaattgtaattttattactgtttggtccataaacacttgtttaccatttccttttttacaagttttaatattttctgcatatataaaacattatttattttgcagtcttttgttgatcacccacccgattggttggaagaagttggtgaaggtcttcgcgagtttttgggccttgaagcgggcccaccgaaaccaaaacccaatcagcagcatcaagatcaagcccgtggtcttgtgctgcctggttataactatctcggacccggaaacggtctcgatcgaggagagcctgtcaacagggcagacgaggtcgcgcgagagcacgacatctcgtacaacgagcagcttgaggcgggagacaacccctacctcaagtacaaccacgcggacgccgagtttcaggagaagctcgccgacgacacatccttcgggggaaacctcggaaaggcagtctttcaggccaagaaaagggttctcgaaccttttggcctggttgaagagggtgctaagacggcccctaccggaaagcggatagacgaccactttccaaaaagaaagaaggctcggaccgaagaggactccaagccttccacctcgtcagacgccgaagctggacccagcggatcccagcagctgcaaatcccagcccaaccagcctcaagtttgggagctgatacaatgtctgcgggaggtggcggcccattgggcgacaataaccaaggtgccgatggagtgggcaatgcctcgggagattggcattgcgattccacgtggatgggggacagagtcgtcaccaagtccacccgaacctgggtgctgcccagctacaacaaccaccagtaccgagagatcaaaagcggctccgtcgacggaagcaacgccaacgcctactttggatacagcaccccctgggggtactttgactttaaccgcttccacagccactggagcccccgagactggcaaagactcatcaacaactactggggcttcagaccccggtccctcagagtcaaaatcttcaacattcaagtcaaagaggtcacggtgcaggactccaccaccaccatcgccaacaacctcacctccaccgtccaagtgtttacggacgacgactaccagctgccctacgtcgtcggcaacgggaccgagggatgcctgccggccttccctccgcaggtctttacgctgccgcagtacggttacgcgacgctgaaccgcgacaacacagaaaatcccaccgagaggagcagcttcttctgcctagagtactttcccagcaagatgctgagaacgggcaacaactttgagtttacctacaactttgaggaggtgcccttccactccagcttcgctcccagtcagaacctcttcaagctggccaacccgctggtggaccagtacttgtaccgcttcgtgagcacaaataacactggcggagtccagttcaacaagaacctggccgggagatacgccaacacctacaaaaactggttcccggggcccatgggccgaacccagggctggaacctgggctccggggtcaaccgcgccagtgtcagcgccttcgccacgaccaataggatggagctcgagggcgcgagttaccaggtgcccccgcagccgaacggcatgaccaacaacctccagggcagcaacacctatgccctggagaacactatgatcttcaacagccagccggcgaacccgggcaccaccgccacgtacctcgagggcaacatgctcatcaccagcgagagcgagacgcagccggtgaaccgcgtggcgtacaacgtcggcgggcagatggccaccaacaaccagagctccaccactgcccccgcgaccggcacgtacaacctccaggaaatcgtgcccggcagcgtgtggatggagagggacgtgtacctccaaggacccatctgggccaagatcccagagacgggggcgcactttcacccctctccggccatgggcggattcggactcaaacacccaccgcccatgatgctcatcaagaacacgcctgtgcccggaaatatcaccagcttctcggacgtgcccgtcagcagcttcatcacccagtacagcaccgggcaggtcaccgtggagatggagtgggagctcaagaaggaaaactccaagaggtggaacccagagatccagtacacaaacaactacaacgacccccagtttgtggactttgccccggacagcaccggggaatacagaagcaccagacctatcggaacccgataccttacccgacccctttaa

SEQ ID NO: 32 - DNA, 2415 bp, Artificial Sequence
  Cap gene expression cassette
gacctttaattcaacccaacacaatatattatagttaaataagaattattatcaaatcatttgtatattaattaaaatactatactgtaaattacattttatttacaatcactcgacgaagacttgatcacccgggtcaggtagtaagtatcgataactttgttttctttcacatttacaactccgacatacaaatcccattacggcagtataaattcgttcattttggatattgtttcagtgtcttttgttgatcacccacccgattggttggaagaagttggtgaaggtcttcgcgagtttttgggccttgaagcgggcccaccgaaaccaaaacccaatcagcagcatcaagatcaagcccgtggtcttgtgctgcctggttataactatctcggacccggaaacggtctcgatcgaggagagcctgtcaacagggcagacgaggtcgcgcgagagcacgacatctcgtacaacgagcagcttgaggcgggagacaacccctacctcaagtacaaccacgcggacgccgagtttcaggagaagctcgccgacgacacatccttcgggggaaacctcggaaaggcagtctttcaggccaagaaaagggttctcgaaccttttggcctggttgaagagggtgctaagacggcccctaccggaaagcggatagacgaccactttccaaaaagaaagaaggctcggaccgaagaggactccaagccttccacctcgtcagacgccgaagctggacccagcggatcccagcagctgcaaatcccagcccaaccagcctcaagtttgggagctgatacaatgtctgcgggaggtggcggcccattgggcgacaataaccaaggtgccgatggagtgggcaatgcctcgggagattggcattgcgattccacgtggatgggggacagagtcgtcaccaagtccacccgaacctgggtgctgcccagctacaacaaccaccagtaccgagagatcaaaagcggctccgtcgacggaagcaacgccaacgcctactttggatacagcaccccctgggggtactttgactttaaccgcttccacagccactggagcccccgagactggcaaagactcatcaacaactactggggcttcagaccccggtccctcagagtcaaaatcttcaacattcaagtcaaagaggtcacggtgcaggactccaccaccaccatcgccaacaacctcacctccaccgtccaagtgtttacggacgacgactaccagctgccctacgtcgtcggcaacgggaccgagggatgcctgccggccttccctccgcaggtctttacgctgccgcagtacggttacgcgacgctgaaccgcgacaacacagaaaatcccaccgagaggagcagcttcttctgcctagagtactttcccagcaagatgctgagaacgggcaacaactttgagtttacctacaactttgaggaggtgcccttccactccagcttcgctcccagtcagaacctcttcaagctggccaacccgctggtggaccagtacttgtaccgcttcgtgagcacaaataacactggcggagtccagttcaacaagaacctggccgggagatacgccaacacctacaaaaactggttcccggggcccatgggccgaacccagggctggaacctgggctccggggtcaaccgcgccagtgtcagcgccttcgccacgaccaataggatggagctcgagggcgcgagttaccaggtgcccccgcagccgaacggcatgaccaacaacctccagggcagcaacacctatgccctggagaacactatgatcttcaacagccagccggcgaacccgggcaccaccgccacgtacctcgagggcaacatgctcatcaccagcgagagcgagacgcagccggtgaaccgcgtggcgtacaacgtcggcgggcagatggccaccaacaaccagagctccaccactgcccccgcgaccggcacgtacaacctccaggaaatcgtgcccggcagcgtgtggatggagagggacgtgtacctccaaggacccatctgggccaagatcccagagacgggggcgcactttcacccctctccggccatgggcggattcggactcaaacacccaccgcccatgatgctcatcaagaacacgcctgtgcccggaaatatcaccagcttctcggacgtgcccgtcagcagcttcatcacccagtacagcaccgggcaggtcaccgtggagatggagtgggagctcaagaaggaaaactccaagaggtggaacccagagatccagtacacaaacaactacaacgacccccagtttgtggactttgccccggacagcaccggggaatacagaagcaccagacctatcggaacccgataccttacccgacccctttaa

SEQ ID NO: 33 - DNA, 2611 bp, Artificial Sequence
  Cap gene expression cassette
gacctttaattcaacccaacacaatatattatagttaaataagaattattatcaaatcatttgtatattaattaaaatactatactgtaaattacattttatttacaatcactcgacgaagacttgatcacccgggtaggacaaggtaagtattcattgtaaatctgatattatttgtattattatacctacctaatttgcagtgcagataaatatgccggatggtaattttattactgtttggtccataaacacttgtttaccatttccttttttacaagttttaatatgttctgcatatataaaacattatgtattttgcagcaccttcaacggctcgggagaagggcggggaagcctcctaacctgcggtgacgttgaggaaaatccgggtccagctgccgacggttatctacccgattggctcgaggacaacctctctgagggcattcgcgagtggtgggcgctgaaacctggagccccgaagcccaaagccaaccagcaaaagcaggacgacggccggggtctggtgcttcctggctacaagtacctcggacccttcaacggactcgacaagggggagcccgtcaacgcggcggacgcagcggccctcgagcacgacaaggcctacgaccagcagctgcaggcgggtgacaatccgtacctgcggtataaccacgccgacgccgagtttcaggagcgtctgcaagaagatacgtcttttgggggcaacctcgggcgagcagtcttccaggccaagaagcgggttctcgaacctctcggtctggttgaggaaggcgctaagacggctcctggaaagaagagaccggtagagccatcaccccagcgttctccagactcctctacgggcatcggcaagaaaggccaacagcccgccagaaaaagactcaattttggtcagactggcgactcagagtcagttccagaccctcaacctctcggagaacctccagcagcgccctctggtgtgggacctaatacaatggctgcaggcggtggcgcaccaatggcagacaataacgaaggcgccgacggagtgggtagttcctcgggaaattggcattgcgattccacatggctgggcgacagagtcatcaccaccagcacccgaacctgggccctgcccacctacaacaaccacctctacaagcaaatctccaacgggacatcgggaggagccaccaacgacaacacctacttcggctacagcaccccctgggggtattttgactttaacagattccactgccacttttcaccacgtgactggcagcgactcatcaacaacaactggggattccggcccaagagactcagcttcaagctcttcaacatccaggtcaaggaggtcacgcagaatgaaggcaccaagaccatcgccaataacctcaccagcaccatccaggtgtttacggactcggagtaccagctgccgtacgttctcggctctgcccaccagggctgcctgcctccgttcccggcggacgtgttcatgattccccagtacggctacctaacactcaacaacggtagtcaggccgtgggacgctcctccttctactgcctggaatactttccttcgcagatgctgagaaccggcaacaacttccagtttacttacaccttcgaggacgtgcctttccacagcagctacgcccacagccagagcttggaccggctgatgaatcctctgattgaccagtacctgtactacttgtctcggactcaaacaacaggaggcacggcaaatacgcagactctgggcttcagccaaggtgggcctaatacaatggccaatcaggcaaagaactggctgccaggaccctgttaccgccaacaacgcgtctcaacgacaaccgggcaaaacaacaatagcaactttgcctggactgctgggaccaaataccatctgaatggaagaaattcattggctaatcctggcatcgctatggcaacacacaaagacgacgaggagcgtttttttcccagtaacgggatcctgatttttggcaaacaaaatgctgccagagacaatgcggattacagcgatgtcatgctcaccagcgaggaagaaatcaaaaccactaaccctgtggctacagaggaatacggtatcgtggcagataacttgcagcagcaaaacacggctcctcaaattggaactgtcaacagccagggggccttacccggtatggtctggcagaaccgggacgtgtacctgcagggtcccatctgggccaagattcctcacacggacggcaacttccacccgtctccgctgatgggcggctttggcctgaaacatcctccgcctcagatcctgatcaagaacacgcctgtacctgcggatcctccgaccaccttcaaccagtcaaagctgaactctttcatcacgcaatacagcaccggacaggtcagcgtggaaattgaatgggagctgcagaaggaaaacagcaagcgctggaaccccgagatccagtacacctccaactactacaaatctacaagtgtggactttgctgttaatacagaaggcgtgtactctgaaccccgccccattggcacccgttacctcacccgtaatctgtaa

SEQ ID NO: 34 - DNA, 2583 bp, Artificial Sequence
  Cap gene expression cassette
gacctttaattcaacccaacacaatatattatagttaaataagaattattatcaaatcatttgtatattaattaaaatactatactgtaaattacattttatttacaatcactcgacgaagacttgatcacccgggggacaaggtaagtattcattgtaaatctgatattatttgtattattatacctacctaatttgcagtgcaggccgccatggtaagtatcgataactttgttttctttcacatttacaactccgacatacaaattgtaattttattactgtttggtccataaacacttgtttaccatttccttttttacaagttttaatattttctgcatatataaaacattatttattttgcaggctgccgacggttatctacccgattggctcgaggacaacctctctgagggcattcgcgagtggtgggcgctgaaacctggagccccgaagcccaaagccaaccagcaaaagcaggacgacggccggggtctggtgcttcctggctacaagtacctcggacccttcaacggactcgacaagggggagcccgtcaacgcggcggacgcagcggccctcgagcacgacaaggcctacgaccagcagctgcaggcgggtgacaatccgtacctgcggtataaccacgccgacgccgagtttcaggagcgtctgcaagaagatacgtcttttgggggcaacctcgggcgagcagtcttccaggccaagaagcgggttctcgaacctctcggtctggttgaggaaggcgctaagacggctcctggaaagaagagaccggtagagccatcaccccagcgttctccagactcctctacgggcatcggcaagaaaggccaacagcccgccagaaaaagactcaattttggtcagactggcgactcagagtcagttccagaccctcaacctctcggagaacctccagcagcgccctctggtgtgggacctaatacaatggctgcaggcggtggcgcaccaatggcagacaataacgaaggcgccgacggagtgggtagttcctcgggaaattggcattgcgattccacatggctgggcgacagagtcatcaccaccagcacccgaacctgggccctgcccacctacaacaaccacctctacaagcaaatctccaacgggacatcgggaggagccaccaacgacaacacctacttcggctacagcaccccctgggggtattttgactttaacagattccactgccacttttcaccacgtgactggcagcgactcatcaacaacaactggggattccggcccaagagactcagcttcaagctcttcaacatccaggtcaaggaggtcacgcagaatgaaggcaccaagaccatcgccaataacctcaccagcaccatccaggtgtttacggactcggagtaccagctgccgtacgttctcggctctgcccaccagggctgcctgcctccgttcccggcggacgtgttcatgattccccagtacggctacctaacactcaacaacggtagtcaggccgtgggacgctcctccttctactgcctggaatactttccttcgcagatgctgagaaccggcaacaacttccagtttacttacaccttcgaggacgtgcctttccacagcagctacgcccacagccagagcttggaccggctgatgaatcctctgattgaccagtacctgtactacttgtctcggactcaaacaacaggaggcacggcaaatacgcagactctgggcttcagccaaggtgggcctaatacaatggccaatcaggcaaagaactggctgccaggaccctgttaccgccaacaacgcgtctcaacgacaaccgggcaaaacaacaatagcaactttgcctggactgctgggaccaaataccatctgaatggaagaaattcattggctaatcctggcatcgctatggcaacacacaaagacgacgaggagcgtttttttcccagtaacgggatcctgatttttggcaaacaaaatgctgccagagacaatgcggattacagcgatgtcatgctcaccagcgaggaagaaatcaaaaccactaaccctgtggctacagaggaatacggtatcgtggcagataacttgcagcagcaaaacacggctcctcaaattggaactgtcaacagccagggggccttacccggtatggtctggcagaaccgggacgtgtacctgcagggtcccatctgggccaagattcctcacacggacggcaacttccacccgtctccgctgatgggcggctttggcctgaaacatcctccgcctcagatcctgatcaagaacacgcctgtacctgcggatcctccgaccaccttcaaccagtcaaagctgaactctttcatcacgcaatacagcaccggacaggtcagcgtggaaattgaatgggagctgcagaaggaaaacagcaagcgctggaaccccgagatccagtacacctccaactactacaaatctacaagtgtggactttgctgttaatacagaaggcgtgtactctgaaccccgccccattggcacccgttacctcacccgtaatctgtaa

SEQ ID NO: 35 - DNA, 2457 bp, Artificial Sequence
  Cap gene expression cassette
gacctttaattcaacccaacacaatatattatagttaaataagaattattatcaaatcatttgtatattaattaaaatactatactgtaaattacattttatttacaatcactcgacgaagacttgatcacccgggtcaggtagtaagtatcgataactttgttttctttcacatttacaactccgacatacaaatcccattacggcagtataaattcgttcattttggatattgtttcagtggctgccgacggttatctacccgattggctcgaggacaacctctctgagggcattcgcgagtggtgggcgctgaaacctggagccccgaagcccaaagccaaccagcaaaagcaggacgacggccggggtctggtgcttcctggctacaagtacctcggacccttcaacggactcgacaagggggagcccgtcaacgcggcggacgcagcggccctcgagcacgacaaggcctacgaccagcagctgcaggcgggtgacaatccgtacctgcggtataaccacgccgacgccgagtttcaggagcgtctgcaagaagatacgtcttttgggggcaacctcgggcgagcagtcttccaggccaagaagcgggttctcgaacctctcggtctggttgaggaaggcgctaagacggctcctggaaagaagagaccggtagagccatcaccccagcgttctccagactcctctacgggcatcggcaagaaaggccaacagcccgccagaaaaagactcaattttggtcagactggcgactcagagtcagttccagaccctcaacctctcggagaacctccagcagcgccctctggtgtgggacctaatacaatggctgcaggcggtggcgcaccaatggcagacaataacgaaggcgccgacggagtgggtagttcctcgggaaattggcattgcgattccacatggctgggcgacagagtcatcaccaccagcacccgaacctgggccctgcccacctacaacaaccacctctacaagcaaatctccaacgggacatcgggaggagccaccaacgacaacacctacttcggctacagcaccccctgggggtattttgactttaacagattccactgccacttttcaccacgtgactggcagcgactcatcaacaacaactggggattccggcccaagagactcagcttcaagctcttcaacatccaggtcaaggaggtcacgcagaatgaaggcaccaagaccatcgccaataacctcaccagcaccatccaggtgtttacggactcggagtaccagctgccgtacgttctcggctctgcccaccagggctgcctgcctccgttcccggcggacgtgttcatgattccccagtacggctacctaacactcaacaacggtagtcaggccgtgggacgctcctccttctactgcctggaatactttccttcgcagatgctgagaaccggcaacaacttccagtttacttacaccttcgaggacgtgcctttccacagcagctacgcccacagccagagcttggaccggctgatgaatcctctgattgaccagtacctgtactacttgtctcggactcaaacaacaggaggcacggcaaatacgcagactctgggcttcagccaaggtgggcctaatacaatggccaatcaggcaaagaactggctgccaggaccctgttaccgccaacaacgcgtctcaacgacaaccgggcaaaacaacaatagcaactttgcctggactgctgggaccaaataccatctgaatggaagaaattcattggctaatcctggcatcgctatggcaacacacaaagacgacgaggagcgtttttttcccagtaacgggatcctgatttttggcaaacaaaatgctgccagagacaatgcggattacagcgatgtcatgctcaccagcgaggaagaaatcaaaaccactaaccctgtggctacagaggaatacggtatcgtggcagataacttgcagcagcaaaacacggctcctcaaattggaactgtcaacagccagggggccttacccggtatggtctggcagaaccgggacgtgtacctgcagggtcccatctgggccaagattcctcacacggacggcaacttccacccgtctccgctgatgggcggctttggcctgaaacatcctccgcctcagatcctgatcaagaacacgcctgtacctgcggatcctccgaccaccttcaaccagtcaaagctgaactctttcatcacgcaatacagcaccggacaggtcagcgtggaaattgaatgggagctgcagaaggaaaacagcaagcgctggaaccccgagatccagtacacctccaactactacaaatctacaagtgtggactttgctgttaatacagaaggcgtgtactctgaaccccgccccattggcacccgttacctcacccgtaatctgtaa

SEQ ID NO: 36 - protein, 18 aa, Thosea asigna virus
EGRGSLLTCGDVEENPGP

SEQ ID NO: 37 - protein, 19 aa, Porcine teschovirus
ATNFSLLKQAGDVEENPGP

SEQ ID NO: 38 - protein, 20 aa, Equine rhinitis A virus
QCTNYALLKLAGDVESNPGP

SEQ ID NO: 39 - protein, 22 aa, Foot-and-mouth disease virus
VKQTLNFDLLKLAGDVESNPGP

SEQ ID NO: 40 - DNA, 10 bp, Artificial Sequence
  The sequence is synthesized.
gtaagtatcg

SEQ ID NO: 41 - DNA, 10 bp, Artificial Sequence
  The sequence is synthesized.
gtaagtattc

SEQ ID NO: 42 - DNA, 20 bp, Artificial Sequence
  The sequence is synthesized.
ccttttcctttttttttcag

SEQ ID NO: 43 - DNA, 20 bp, Artificial Sequence
  The sequence is synthesized.
aaacattatttattttgcag

SEQ ID NO: 44 - DNA, 20 bp, Artificial Sequence
  The sequence is synthesized.
cattttggatattgtttcag

SEQ ID NO: 45 - DNA, 21 bp, Artificial Sequence
  Q-ITR-F
ggaacccctagtgatggagtt

SEQ ID NO: 46 - DNA, 16 bp, Artificial Sequence
  Q-ITR-R
cggcctcagtgagcga